European Patent Specification EP 3 457 840 B1, published April 10, 2024. Title: METHODS FOR BREAKING IMMUNOLOGICAL TOLERANCE USING MULTIPLE GUIDE RNAS. Applicant: Regeneron Pharmaceuticals, Inc. The sequence listing filed with the application follows.

SEQUENCE LISTING (152 sequences)

SEQ ID NO: 1 - DNA, 23 bp, Artificial Sequence
  Guide RNA recognition sequence
  misc_feature (2)...(21): n = A, T, C, or G
gnnnnnnnnnnnnnnnnnnnngg

SEQ ID NO: 2 - DNA, 23 bp, Artificial Sequence
  Guide RNA recognition sequence
  misc_feature (1)...(21): n = A, T, C, or G
nnnnnnnnnnnnnnnnnnnnngg

SEQ ID NO: 3 - DNA, 25 bp, Artificial Sequence
  Guide RNA recognition sequence
  misc_feature (3)...(23): n = A, T, C, or G
ggnnnnnnnnnnnnnnnnnnnnngg

SEQ ID NO: 4 - DNA, 20 bp, Artificial Sequence
  C5 (Hc) gRNA A DNA-targeting segment (100 bp from target locus endpoint)
atcacaaaccagttaaccgg

SEQ ID NO: 5 - DNA, 20 bp, Artificial Sequence
  C5 (Hc) gRNA B DNA-targeting segment (500 bp from target locus endpoint)
tttcagacgagccgacccgg

SEQ ID NO: 6 - DNA, 20 bp, Artificial Sequence
  C5 (Hc) gRNA C DNA-targeting segment (38200 and 37500 bp from target locus endpoints)
tgtgtgtcatagcgatgtcg

SEQ ID NO: 7 - DNA, 20 bp, Artificial Sequence
  C5 (Hc) gRNA D DNA-targeting segment (43500 and 32200 bp from target locus endpoints)
aacaggtaccctatcctcac

SEQ ID NO: 8 - DNA, 20 bp, Artificial Sequence
  C5 (Hc) gRNA E DNA-targeting segment (500 bp from target locus endpoint)
ggcccggacctagtctctct

SEQ ID NO: 9 - DNA, 20 bp, Artificial Sequence
  C5 (Hc) gRNA E2 DNA-targeting segment (100 bp from target locus endpoint)
tcgtggttgcatgcgcactg

SEQ ID NO: 10 - DNA, 20 bp, Artificial Sequence
  Lrp5 gRNA A DNA-targeting segment (50 bp from target locus end point)
gggaacccacagcatactcc

SEQ ID NO: 11 - DNA, 20 bp, Artificial Sequence
  Lrp5 gRNA B DNA-targeting segment (500 bp from target locus end point)
gaatcatgcacggctacccc

SEQ ID NO: 12 - DNA, 20 bp, Artificial Sequence
  Lrp5 gRNA B2 DNA-targeting segment (1000 bp from target locus end point)
tgctcctatggggaggcgcg

SEQ ID NO: 13 - DNA, 20 bp, Artificial Sequence
  Lrp5 gRNA C DNA-targeting segment (29900 and 38430 bp from target locus end points)
actgagatcaatgaccccga

SEQ ID NO: 14 - DNA, 20 bp, Artificial Sequence
  Lrp5 gRNA D DNA-targeting segment (29950 and 38380 bp from target locus end points)
gggtcgcccggaacctctac

SEQ ID NO: 15 - DNA, 20 bp, Artificial Sequence
  Lrp5 gRNA E2 DNA-targeting segment (1000 bp from target locus end point)
cttggataacattgataccc

SEQ ID NO: 16 - DNA, 20 bp, Artificial Sequence
  Lrp5 gRNA E DNA-targeting segment (500 bp from target locus end point)
ggggcagagcccttatatca

SEQ ID NO: 17 - DNA, 20 bp, Artificial Sequence
  Lrp5 gRNA F DNA-targeting segment (50 bp from target locus end point)
tcgctcacattaatccctag

SEQ ID NO: 18 - DNA, 20 bp, Artificial Sequence
  Ror1 gRNA A DNA-targeting segment (200 bp from target locus end point)
tgtgggcctttgctgatcac

SEQ ID NO: 19 - DNA, 20 bp, Artificial Sequence
  Ror1 gRNA B DNA-targeting segment (1000 bp from target locus end point)
aatctatgatcctatggcct

SEQ ID NO: 20 - DNA, 20 bp, Artificial Sequence
  Ror1 gRNA D DNA-targeting segment (54300 and 55500 bp from target locus end points)
tgccaatagcagtgacttga

SEQ ID NO: 21 - DNA, 20 bp, Artificial Sequence
  Ror1 gRNA C DNA-targeting segment (54500 and 55300 bp from target locus end points)
gggaagaatgggctattgtc

SEQ ID NO: 22 - DNA, 20 bp, Artificial Sequence
  Ror1 gRNA E DNA-targeting segment (1000 bp from target locus end point)
ggttgtttgtgctgatgacg

SEQ ID NO: 23 - DNA, 20 bp, Artificial Sequence
  Ror1 gRNA F DNA-targeting segment (200 bp from target locus end point)
ccgtcctaggccttctacgt

SEQ ID NO: 24 - DNA, 20 bp, Artificial Sequence
  Trpa1 gRNA A DNA-targeting segment (100 bp from target locus end point)
gtactggggaatcggtggtc

SEQ ID NO: 25 - DNA, 20 bp, Artificial Sequence
  Trpa1 gRNA A2 DNA-targeting segment (500 bp from target locus end point)
cacgcactccaaatttatcc

SEQ ID NO: 26 - DNA, 20 bp, Artificial Sequence
  Trpa1 gRNA B DNA-targeting segment (1000 bp from target locus end point)
ctaagtgtgtatcagtacat

SEQ ID NO: 27 - DNA, 20 bp, Artificial Sequence
  Trpa1 gRNA C DNA-targeting segment (25600 and 19740 bp from target locus end points)
tgccctgcacaataagcgca

SEQ ID NO: 28 - DNA, 20 bp, Artificial Sequence
  Trpa1 gRNA D DNA-targeting segment (26970 and 18370 bp from target locus end points)
actcattgaaacgttatggc

SEQ ID NO: 29 - DNA, 20 bp, Artificial Sequence
  Trpa1 gRNA E2 DNA-targeting segment (1000 bp from target locus end point)
agtaagggtggattaaattc

SEQ ID NO: 30 - DNA, 20 bp, Artificial Sequence
  Trpa1 gRNA E DNA-targeting segment (500 bp from target locus end point)
gccatctagattcatgtaac

SEQ ID NO: 31 - DNA, 20 bp, Artificial Sequence
  Trpa1 gRNA F DNA-targeting segment (100 bp from target locus end point)
gactagaaatgttctgcacc

SEQ ID NO: 32 - DNA, 21 bp, Artificial Sequence
  190045 forward primer
gagctcatagccaacagcttg

SEQ ID NO: 33 - DNA, 20 bp, Artificial Sequence
  190061 forward primer
atgcatcagatcacgctcag

SEQ ID NO: 34 - DNA, 20 bp, Artificial Sequence
  190068 forward primer
gtccttgtggcatttccaac

SEQ ID NO: 35 - DNA, 24 bp, Artificial Sequence
  190030 forward primer
ccagtatggtgtcagttaatagcg

SEQ ID NO: 36 - DNA, 19 bp, Artificial Sequence
  190033 forward primer (same as forward primer for SV 48.3 in Fig. 6)
ctgtgcagaaagcagcctc

SEQ ID NO: 37 - DNA, 20 bp, Artificial Sequence
  190013 forward primer
cctctccctctaggcacctg

SEQ ID NO: 38 - DNA, 20 bp, Artificial Sequence
  190045 reverse primer
tctttaagggctccgttgtc

SEQ ID NO: 39 - DNA, 20 bp, Artificial Sequence
  190061 reverse primer
aagaccaaccattcacccag

SEQ ID NO: 40 - DNA, 20 bp, Artificial Sequence
  190068 reverse primer
ttcccagtccaagtcaaagg

SEQ ID NO: 41 - DNA, 20 bp, Artificial Sequence
  190030 reverse primer
ctgttatctgcaaggcaccc

SEQ ID NO: 42 - DNA, 20 bp, Artificial Sequence
  190033 reverse primer (same as reverse primer for SV 48.3 in Fig. 6)
acaactggatcctgattcgc

SEQ ID NO: 43 - DNA, 20 bp, Artificial Sequence
  190013 reverse primer
taagagggcatgggtgagac

SEQ ID NO: 44 - DNA, 20 bp, Artificial Sequence
  C2 probe (B6) - SNV 0.32 in Fig. 6
aattcagaagacctatcgta

SEQ ID NO: 45 - DNA, 21 bp, Artificial Sequence
  T3 probe (B6) - SNV 1.2 in Fig. 6
tatgtgtataggtgtttggat

SEQ ID NO: 46 - DNA, 19 bp, Artificial Sequence
  T6 probe (B6) - SNV 11.1 in Fig. 6
tacattgctaaatgaaacc

SEQ ID NO: 47 - DNA, 16 bp, Artificial Sequence
  T7 probe (B6) - SNV 13.2 in Fig. 6
cgcagtcatgcacata

SEQ ID NO: 48 - DNA, 20 bp, Artificial Sequence
  T8 probe (B6) - SNV 17.5 in Fig. 6
ttataaagcccagtatgtac

SEQ ID NO: 49 - DNA, 14 bp, Artificial Sequence
  T9 probe (B6) - SNV 25.8 in Fig. 6
tgctgcataatcag

SEQ ID NO: 50 - DNA, 18 bp, Artificial Sequence
  T10 probe (B6) - SNV 33.0 in Fig. 6
tcaggagtgaattggata

SEQ ID NO: 51 - DNA, 16 bp, Artificial Sequence
  T11 probe (B6) - SNV 38.3 in Fig. 6
ctgctacttacctttg

SEQ ID NO: 52 - DNA, 13 bp, Artificial Sequence
  T13 probe (B6) - SNV 49.6 in Fig. 6
aggaggaaaacgc

SEQ ID NO: 53 - DNA, 17 bp, Artificial Sequence
  T14 probe (B6) - SNV 57.2 in Fig. 6
cctttgttcctcataag

SEQ ID NO: 54 - DNA, 20 bp, Artificial Sequence
  C2 probe (129) - SNV 0.32 in Fig. 6
aattcagaagacctattgta

SEQ ID NO: 55 - DNA, 21 bp, Artificial Sequence
  T3 probe (129) - SNV 1.2 in Fig. 6
tatgtgtataggtgtttgcat

SEQ ID NO: 56 - DNA, 16 bp, Artificial Sequence
  T6 probe (129) - SNV 11.1 in Fig. 6
cattgctacatgaaac

SEQ ID NO: 57 - DNA, 16 bp, Artificial Sequence
  T7 probe (129) - SNV 13.2 in Fig. 6
cgcagtcatgcacgta

SEQ ID NO: 58 - DNA, 23 bp, Artificial Sequence
  T8 probe (129) - SNV 17.5 in Fig. 6
tgagaatttataaagcccaatat

SEQ ID NO: 59 - DNA, 14 bp, Artificial Sequence
  T9 probe (129) - SNV 25.8 in Fig. 6
tgctgcatgatcag

SEQ ID NO: 60 - DNA, 15 bp, Artificial Sequence
  T10 probe (129) - SNV 33.0 in Fig. 6
tcaggagtgaatcgg

SEQ ID NO: 61 - DNA, 16 bp, Artificial Sequence
  T11 probe (129) - SNV 38.3 in Fig. 6
ctgctagttacctttg

SEQ ID NO: 62 - DNA, 15 bp, Artificial Sequence
  T13 probe (129) - SNV 49.6 in Fig. 6
aggaggaagacgcag

SEQ ID NO: 63 - DNA, 17 bp, Artificial Sequence
  T14 probe (129) - SNV 57.2 in Fig. 6
ctttgttcttcataagc

SEQ ID NO: 64 - DNA, 25 bp, Artificial Sequence
  C2 forward primer - SNV 0.32 in Fig. 6
atgagggatttccttaatcagacaa

SEQ ID NO: 65 - DNA, 29 bp, Artificial Sequence
  T3 forward primer - SNV 1.2 in Fig. 6
tggtatgtttattcttactcaaggttttg

SEQ ID NO: 66 - DNA, 22 bp, Artificial Sequence
  T6 forward primer - SNV 11.1 in Fig. 6
gggcaactgatggaaagaactc

SEQ ID NO: 67 - DNA, 23 bp, Artificial Sequence
  T7 forward primer - SNV 13.2 in Fig. 6
gactgacgcacaaacttgtcctt

SEQ ID NO: 68 - DNA, 26 bp, Artificial Sequence
  T8 forward primer - SNV 17.5 in Fig. 6
cccaaagcatataacaagaacaaatg

SEQ ID NO: 69 - DNA, 18 bp, Artificial Sequence
  T9 forward primer - SNV 25.8 in Fig. 6
gcaggacgcaggcgttta

SEQ ID NO: 70 - DNA, 23 bp, Artificial Sequence
  T10 forward primer - SNV 33.0 in Fig. 6
gcatcctcatggcagtctacatc

SEQ ID NO: 71 - DNA, 20 bp, Artificial Sequence
  T11 forward primer - SNV 38.3 in Fig. 6
cctgccccttgatgagtgtt

SEQ ID NO: 72 - DNA, 23 bp, Artificial Sequence
  T13 forward primer - SNV 49.6 in Fig. 6
ccctctttgatatgctcgtgtgt

SEQ ID NO: 73 - DNA, 22 bp, Artificial Sequence
  T14 forward primer - SNV 57.2 in Fig. 6
tcccacaggtccatgtctttaa

SEQ ID NO: 74 - DNA, 28 bp, Artificial Sequence
  C2 reverse primer - SNV 0.32 in Fig. 6
agactacaatgagctaccatcataaggt

SEQ ID NO: 75 - DNA, 24 bp, Artificial Sequence
  T3 reverse primer - SNV 1.2 in Fig. 6
caaccatctaaaactccagttcca

SEQ ID NO: 76 - DNA, 28 bp, Artificial Sequence
  T6 reverse primer - SNV 11.1 in Fig. 6
tgtgtaacaggacagttgaatgtagaga

SEQ ID NO: 77 - DNA, 19 bp, Artificial Sequence
  T7 reverse primer - SNV 13.2 in Fig. 6
cttaaaacccgccctgcat

SEQ ID NO: 78 - DNA, 26 bp, Artificial Sequence
  T8 reverse primer - SNV 17.5 in Fig. 6
ctacaggagatgtggctgttctatgt

SEQ ID NO: 79 - DNA, 22 bp, Artificial Sequence
  T9 reverse primer - SNV 25.8 in Fig. 6
tcagcgtgattcgcttgtagtc

SEQ ID NO: 80 - DNA, 26 bp, Artificial Sequence
  T10 reverse primer - SNV 33.0 in Fig. 6
tgcatagctgtttgaataatgacaag

SEQ ID NO: 81 - DNA, 21 bp, Artificial Sequence
  T11 reverse primer - SNV 38.3 in Fig. 6
tgcagcatctctgtcaagcaa

SEQ ID NO: 82 - DNA, 24 bp, Artificial Sequence
  T13 reverse primer - SNV 49.6 in Fig. 6
gcaacaacataacccacagcataa

SEQ ID NO: 83 - DNA, 23 bp, Artificial Sequence
  T14 reverse primer - SNV 57.2 in Fig. 6
gctaagcgtttggaagaaattcc

SEQ ID NO: 84 - DNA, 20 bp, Artificial Sequence
  Forward primer for SV 13.7 in Fig. 6
taggctctaaggatgctggc

SEQ ID NO: 85 - DNA, 20 bp, Artificial Sequence
  Reverse primer for SV 13.7 in Fig. 6
aagcagcttcaaaccctctg

SEQ ID NO: 86 - DNA, 20 bp, Artificial Sequence
  Forward primer for SV 20.0 in Fig. 6
ttacttggccttggaactgc

SEQ ID NO: 87 - DNA, 21 bp, Artificial Sequence
  Reverse primer for SV 20.0 in Fig. 6
tgattcgtaatcgtcactgcc

SEQ ID NO: 88 - DNA, 20 bp, Artificial Sequence
  Forward primer for SV 36.9 in Fig. 6
tcctgtcccgagaaactgtc

SEQ ID NO: 89 - DNA, 20 bp, Artificial Sequence
  Reverse primer for SV 36.9 in Fig. 6
agctggctttcagagagctg

SEQ ID NO: 90 - DNA, 20 bp, Artificial Sequence
  Forward primer for SV 56.7 in Fig. 6
ttagaaagtgccaaccaggc

SEQ ID NO: 91 - DNA, 20 bp, Artificial Sequence
  Reverse primer for SV 56.7 in Fig. 6
ctctggctaggaacaatggc

SEQ ID NO: 92 - DNA, 25 bp, Artificial Sequence
  m-lr-f primer for Lrp5 locus
gttaggtgcagggtctactcagctg

SEQ ID NO: 93 - DNA, 20 bp, Artificial Sequence
  m-5'-f primer for Lrp5 locus
ggaggagaggagaagcagcc

SEQ ID NO: 94 - DNA, 20 bp, Artificial Sequence
  m-A primer for Lrp5 locus
ggaggagaggagaagcagcc

SEQ ID NO: 95 - DNA, 26 bp, Artificial Sequence
  h-lr-r primer for Lrp5 locus
gcaaacagccttcttcccacattcgg

SEQ ID NO: 96 - DNA, 24 bp, Artificial Sequence
  m-5'-r primer for Lrp5 locus
ttgctttcagtagttcaggtgtgc

SEQ ID NO: 97 - DNA, 20 bp, Artificial Sequence
  h-5'-r primer for Lrp5 locus
ggcgttgtcaggaagttgcc

SEQ ID NO: 98 - DNA, 22 bp, Artificial Sequence
  m-F primer for Lrp5 locus
tgaagttgagaggcacatgagg

SEQ ID NO: 99 - DNA, 24 bp, Artificial Sequence
  m-E2 primer for Lrp5 locus
tagagtagccacaggcagcaaagc

SEQ ID NO: 100 - DNA, 22 bp, Artificial Sequence
  7064retU forward primer
cctcctgagctttcctttgcag

SEQ ID NO: 101 - DNA, 25 bp, Artificial Sequence
  7064retU reverse primer
cctagacaacacagacactgtatca

SEQ ID NO: 102 - DNA, 23 bp, Artificial Sequence
  7064retU TAQMAN probe
ttctgcccttgaaaaggagaggc

SEQ ID NO: 103 - DNA, 18 bp, Artificial Sequence
  7064retD forward primer
cctctgaggccacctgaa

SEQ ID NO: 104 - DNA, 23 bp, Artificial Sequence
  7064retD reverse primer
ccctgacaagttctgccttctac

SEQ ID NO: 105 - DNA, 21 bp, Artificial Sequence
  7064retD TAQMAN probe
tgcccaagcctctgcagcttt

SEQ ID NO: 106 - DNA, 19 bp, Artificial Sequence
  7140retU forward primer
cccagcatctgacgacacc

SEQ ID NO: 107 - DNA, 21 bp, Artificial Sequence
  7140retU reverse primer
gaccactgtgggcatctgtag

SEQ ID NO: 108 - DNA, 27 bp, Artificial Sequence
  7140retU TAQMAN probe
ccgagtctgctgttactgttagcatca

SEQ ID NO: 109 - DNA, 20 bp, Artificial Sequence
  7140retD forward primer
cccgacaccttctgagcatg

SEQ ID NO: 110 - DNA, 21 bp, Artificial Sequence
  7140retD reverse primer
tgcaggctgagtcaggatttg

SEQ ID NO: 111 - DNA, 25 bp, Artificial Sequence
  7140retD TAQMAN probe
tagtcacgttttgtgacaccccaga

SEQ ID NO: 112 - DNA, 20 bp, Artificial Sequence
  Folh1 gRNA A DNA-targeting segment
tgaaccaattgtgtagcctt

SEQ ID NO: 113 - DNA, 20 bp, Artificial Sequence
  Folh1 gRNA A2 DNA-targeting segment
aatagtggtaaagcaccatg

SEQ ID NO: 114 - DNA, 20 bp, Artificial Sequence
  Folh1 gRNA B DNA-targeting segment
gtgtgctaaggatcgaagtc

SEQ ID NO: 115 - DNA, 20 bp, Artificial Sequence
  Folh1 gRNA C DNA-targeting segment
caccgagatgcttgggtatt

SEQ ID NO: 116 - DNA, 20 bp, Artificial Sequence
  Folh1 gRNA D DNA-targeting segment
tgtaaccgccctgaatgacc

SEQ ID NO: 117 - DNA, 20 bp, Artificial Sequence
  Folh1 gRNA E DNA-targeting segment
aaaagggcatcataaatccc

SEQ ID NO: 118 - DNA, 20 bp, Artificial Sequence
  Folh1 gRNA E2 DNA-targeting segment
tcaaaaatagtcatacacct

SEQ ID NO: 119 - DNA, 20 bp, Artificial Sequence
  Folh1 gRNA F DNA-targeting segment
ggtctctagtacattgtaga

SEQ ID NO: 120 - DNA, 20 bp, Artificial Sequence
  Adamts5 gRNA A DNA-targeting segment
ggtggtggtgctgacggaca

SEQ ID NO: 121 - DNA, 20 bp, Artificial Sequence
  Adamts5 gRNA A2 DNA-targeting segment
tatgagatcaacactcgcta

SEQ ID NO: 122 - DNA, 20 bp, Artificial Sequence
  Adamts5 gRNA B DNA-targeting segment
ccaaggacttccccacgtta

SEQ ID NO: 123 - DNA, 20 bp, Artificial Sequence
  Adamts5 gRNA C DNA-targeting segment
tgcttcccttatgcaagatt

SEQ ID NO: 124 - DNA, 20 bp, Artificial Sequence
  Adamts5 gRNA D DNA-targeting segment
ttaggtaccctatttgaata

SEQ ID NO: 125 - DNA, 20 bp, Artificial Sequence
  Adamts5 gRNA E2 DNA-targeting segment
tgcagtgggtgacaggtcca

SEQ ID NO: 126 - DNA, 20 bp, Artificial Sequence
  Adamts5 gRNA E DNA-targeting segment
agggttatactgacgttgtg

SEQ ID NO: 127 - DNA, 20 bp, Artificial Sequence
  Adamts5 gRNA F DNA-targeting segment
tgtctttcaaggagggctac

SEQ ID NO: 128 - DNA, 20 bp, Artificial Sequence
  Dpp4 gRNA A DNA-targeting segment
actagtagacctgaggggtt

SEQ ID NO: 129 - DNA, 20 bp, Artificial Sequence
  Dpp4 gRNA B DNA-targeting segment
gctccagtgtttaggccttg

SEQ ID NO: 130 - DNA, 20 bp, Artificial Sequence
  Dpp4 gRNA B2 DNA-targeting segment
ggcaagctgaaaacgcatgc

SEQ ID NO: 131 - DNA, 20 bp, Artificial Sequence
  Dpp4 gRNA C DNA-targeting segment
gtagatcgctttccactacc

SEQ ID NO: 132 - DNA, 20 bp, Artificial Sequence
  Dpp4 gRNA D DNA-targeting segment
gaactccactgctcgtgagc

SEQ ID NO: 133 - DNA, 20 bp, Artificial Sequence
  Dpp4 gRNA E2 DNA-targeting segment
ataggtgggcactattgaag

SEQ ID NO: 134 - DNA, 20 bp, Artificial Sequence
  Dpp4 gRNA E DNA-targeting segment
atgggaaggtttataccagc

SEQ ID NO: 135 - DNA, 20 bp, Artificial Sequence
  Dpp4 gRNA F DNA-targeting segment
cggtgtaaaaacaacgggaa

SEQ ID NO: 136 - DNA, 20 bp, Artificial Sequence
  Forward primer for SV 6.1 in Fig. 8
ggaatgccaaggctactgtc

SEQ ID NO: 137 - DNA, 20 bp, Artificial Sequence
  Reverse primer for SV 6.1 in Fig. 8
aaaagtctgctttgggtggt

SEQ ID NO: 138 - DNA, 21 bp, Artificial Sequence
  Forward primer for SV 6.3 in Fig. 8
cttcatgaacctcactcagga

SEQ ID NO: 139 - DNA, 21 bp, Artificial Sequence
  Reverse primer for SV 6.3 in Fig. 8
tctcggagtcaggatttacct

SEQ ID NO: 140 - DNA, 20 bp, Artificial Sequence
  Forward primer for SV 7.8 in Fig. 8
tgtctctttgcctgttgctg

SEQ ID NO: 141 - DNA, 22 bp, Artificial Sequence
  Reverse primer for SV 7.8 in Fig. 8
tctgctctacaaggcttacgtg

SEQ ID NO: 142 - DNA, 20 bp, Artificial Sequence
  Forward primer for SV 16 in Fig. 8
caaccaggcagacttacagc

SEQ ID NO: 143 - DNA, 20 bp, Artificial Sequence
  Reverse primer for SV 16 in Fig. 8
ggcctaggaaccagtcaaaa

SEQ ID NO: 144 - DNA, 23 bp, Artificial Sequence
  Forward primer for SV 25.5 in Fig. 8
gcttactggaaagctacataggg

SEQ ID NO: 145 - DNA, 22 bp, Artificial Sequence
  Reverse primer for SV 25.5 in Fig. 8
caacaacatagaaacccctgtc

SEQ ID NO: 146 - DNA, 6 bp, Artificial Sequence
  S. aureus Cas9 PAM sequence
  misc_feature (1)...(2): n = A, T, C, or G
  misc_feature (4)...(5): r = A or G
nngrrt

SEQ ID NO: 147 - DNA, 5 bp, Artificial Sequence
  S. aureus Cas9 PAM sequence
  misc_feature (1)...(2): n = A, T, C, or G
  misc_feature (4)...(5): r = A or G
nngrr

SEQ ID NO: 148 - DNA, 3155 bp, Artificial Sequence
  Engineered Human Vk1-39Jk5 Locus
ggcgcgccgtagctttgaattttaaacatctatttgacaagaaatgcatagttccttctctttaaaataatgtaatgtttctttcaagaataagcttggtttgatgcctctctccccaacatgatagaagtgtagcataaatctatgaaaaattccatttccctgtgcctacaacaactacctgggattgaaaacttcttcccttgctctagtcctttcttctacacctacttccacatcatctgtgactcaaaacaatacttgtcaggaaagatcccggaaagagcaaaaaagacttccttagaggtgtcagagattcctatgccactatctgtcatctctagaaggggttgtgagtatgaggaagagcagagcttgtaaattttctacttgctttgacttccactgtatttcctaacaacaacaaccacagcaacacccataacatcacaggacaaacttctagtacttccaaggctttagtctcagtaaatcttctctacctccatcacagcagctagaaggtttgatactcatacaaatagtactgtagctttctgttcataattggaaaaatagacaagacccaatgtaatacaggctttccttcagccagttagcgttcagtttttggatcaccattgcacacatatacccagcatatgtctaatatatatgtagaaatccgtgaagcaagagttataatagcttgtgttttctattgtattgtattttcctcttatatcatcttcttcttcgttcattaaaaaaaaaccgttcaagtaggtctaaattaattattggatcataagtagataaaatattttatttcataacacattgacccgatgaatatgtttctttgccagacatagtcctcatttccaaggtaacaagcctgaaaaaattatactggagcaagtcaacaggtaatgatggtagcttttccttattgtcctggggcaagaataagacaaaagataacagggtagaataaagattgtgtaagaaagaaggacagcaacaggacatgggaaccttttatagagtaacattttgataatggatgatgagaattaatgagttagacagggatgggtgggaatgattgaaggtgtgagtactttagcacagattaagaccaaatcattaggatttaaagagttgtgtagagttagtgaaggaaaagccttagaattaaatttggctgcggataaaacattcttggattagactgaagactcttttctgtgctaagtaagtatatttatgataatgatgatgactgtagtgctgaatatttaataaataaaaacaaaattaattgccgcatacataatgtcctgaatactattgtaaatgttttatcttatttcctttaaactgtctacagcactataaggtaggtaccagtattgtcacagttacacagatatggaaaccgagacacagggaagttaagttacttgatcaatttcaagcaatcggcaagccatggagcatctatgtcagggctgccaggacatgtgactgtaaacagaagtttttcactttttaactcaaagagggtatgtggctgggttaatggaaagcttcaggaccctcagaaaacattactaacaagcaaatgaaaggtgtatctggaagattaagttttaacagactcttcatttccatcgatccaataatgcacttagggagatgactgggcatattgaggataggaagagagaagtgaaaacacagctttttatattgttcttaacaggcttgtgccaaacatcttctgggtggatttaggtgattgaggagaagaaagacacaggagcgaaattctctgagcacaagggaggagttctacactcagactgagccaacagacttttctggcctgacaaccagggcggcgcaggatgctcagtgcagagaggaagaagcaggtggtctttgcagctgaaagctcagctgatttgcatatggagtcattatacaacatcccagaattctttaagggcagctgccaggaagctaagaagcatcctctcttctagctctcagagatggagacagacacactcctgctatgggtgctgctgctctgggttccaggtgagggtacagataagtgttatgagcaacctctgtggccattatgatgctccatgcctctctgttcttgatcactataattagggcatttgtcactggttttaagtttccccagtcccctgaattttccattttctcagagtgatgtccaaaattattcttaaaaatttaaatgaaaaggtcctctgctgtgaaggcttttaaagatatataaaaataatctttgtgtttatcattccaggtgccagatgtgacatccagatgacccagtctccatcctccctgtctgcatctgtaggagacagagtcaccatcacttgccgggcaagtcagagcattagcagctatttaaattggtatcagcagaaaccagggaaagcccctaagctcctgatctatgctgcatccagtttgcaaagtggggtcccatcaaggttcagtggcagtggatctgggacagatttcactctcaccatcagcagtctgcaacctgaagattttgcaacttactactgtcaacagagttacagtacccctccgatcaccttcggccaagggacacgactggagattaaacgtaagtaatttttcactattgtcttctgaaatttgggtctgatggccagtattgacttttagaggcttaaataggagtttggtaaagattggtaaatgagggcatttaagatttgccatgggttgcaaaagttaaactcagcttcaaaaatggatttggagaaaaaaagattaaattgctctaaactgaatgacacaaagtaaaaaaaaaaagtgtaactaaaaaggaacccttgtatttctaaggagcaaaagtaaatttatttttgttcactcttgccaaatattgtattggttgttgctgattatgcatgatacagaaaagtggaaaaatacattttttagtctttctcccttttgtttgataaattattttgtcagacaacaataaaaatcaatagcacgccctaagatctagatgcatgctcgagtgccatttcattacctctttctccgcacccgacatagat

SEQ ID NO: 149 - DNA, 3166 bp, Artificial Sequence
  Engineered Human Vk3-20Jk1 Locus
ggcgcgccgtagctttgaattttaaacatctatttgacaagaaatgcatagttccttctctttaaaataatgtaatgtttctttcaagaataagcttggtttgatgcctctctccccaacatgatagaagtgtagcataaatctatgaaaaattccatttccctgtgcctacaacaactacctgggattgaaaacttcttcccttgctctagtcctttcttctacacctacttccacatcatctgtgactcaaaacaatacttgtcaggaaagatcccggaaagagcaaaaaagacttccttagaggtgtcagagattcctatgccactatctgtcatctctagaaggggttgtgagtatgaggaagagcagagcttgtaaattttctacttgctttgacttccactgtatttcctaacaacaacaaccacagcaacacccataacatcacaggacaaacttctagtacttccaaggctttagtctcagtaaatcttctctacctccatcacagcagctagaaggtttgatactcatacaaatagtactgtagctttctgttcataattggaaaaatagacaagacccaatgtaatacaggctttccttcagccagttagcgttcagtttttggatcaccattgcacacatatacccagcatatgtctaatatatatgtagaaatccgtgaagcaagagttataatagcttgtgttttctattgtattgtattttcctcttatatcatcttcttcttcgttcattaaaaaaaaaccgttcaagtaggtctaaattaattattggatcataagtagataaaatattttatttcataacacattgacccgatgaatatgtttctttgccagacatagtcctcatttccaaggtaacaagcctgaaaaaattatactggagcaagtcaacaggtaatgatggtagcttttccttattgtcctggggcaagaataagacaaaagataacagggtagaataaagattgtgtaagaaagaaggacagcaacaggacatgggaaccttttatagagtaacattttgataatggatgatgagaattaatgagttagacagggatgggtgggaatgattgaaggtgtgagtactttagcacagattaagaccaaatcattaggatttaaagagttgtgtagagttagtgaaggaaaagccttagaattaaatttggctgcggataaaacattcttggattagactgaagactcttttctgtgctaagtaagtatatttatgataatgatgatgactgtagtgctgaatatttaataaataaaaacaaaattaattgccgcatacataatgtcctgaatactattgtaaatgttttatcttatttcctttaaactgtctacagcactataaggtaggtaccagtattgtcacagttacacagatatggaaaccgagacacagggaagttaagttacttgatcaatttcaagcaatcggcaagccatggagcatctatgtcagggctgccaggacatgtgactgtaaacagaagtttttcactttttaactcaaagagggtatgtggctgggttaatggaaagcttcaggaccctcagaaaacattactaacaagcaaatgaaaggtgtatctggaagattaagttttaacagactcttcatttccatcgatccaataatgcacttagggagatgactgggcatattgaggataggaagagagaagtgaaaacacagctttttatattgttcttaacaggcttgtgccaaacatcttctgggtggatttaggtgattgaggagaagaaagacacaggagcgaaattctctgagcacaagggaggagttctacactcagactgagccaacagacttttctggcctgacaaccagggcggcgcaggatgctcagtgcagagaggaagaagcaggtggtctttgcagctgaaagctcagctgatttgcatatggagtcattatacaacatcccagaattctttaagggcagctgccaggaagctaagaagcatcctctcttctagctctcagagatggagacagacacactcctgctatgggtgctgctgctctgggttccaggtgagggtacagataagtgttatgagcaacctctgtggccattatgatgctccatgcctctctgttcttgatcactataattagggcatttgtcactggttttaagtttccccagtcccctgaattttccattttctcagagtgatgtccaaaattattcttaaaaatttaaatgaaaaggtcctctgctgtgaaggcttttaaagatatataaaaataatctttgtgtttatcattccaggtgccagatgtataccaccggagaaattgtgttgacgcagtctccaggcaccctgtctttgtctccaggggaaagagccaccctctcctgcagggccagtcagagtgttagcagcagctacttagcctggtaccagcagaaacctggccaggctcccaggctcctcatctatggtgcatccagcagggccactggcatcccagacaggttcagtggcagtgggtctgggacagacttcactctcaccatcagcagactggagcctgaagattttgcagtgtattactgtcagcagtatggtagctcaccttggacgttcggccaagggaccaaggtggaaatcaaacgtaagtaatttttcactattgtcttctgaaatttgggtctgatggccagtattgacttttagaggcttaaataggagtttggtaaagattggtaaatgagggcatttaagatttgccatgggttgcaaaagttaaactcagcttcaaaaatggatttggagaaaaaaagattaaattgctctaaactgaatgacacaaagtaaaaaaaaaaagtgtaactaaaaaggaacccttgtatttctaaggagcaaaagtaaatttatttttgttcactcttgccaaatattgtattggttgttgctgattatgcatgatacagaaaagtggaaaaatacattttttagtctttctcccttttgtttgataaattattttgtcagacaacaataaaaatcaatagcacgccctaagatctagatgcatgctcgagtgccatttcattacctctttctccgcacccgacatagat

SEQ ID NO: 150 - DNA, 82 bp, Artificial Sequence
  Guide RNA Scaffold v1
gttggaaccattcaaaacagcatagcaagttaaaataaggctagtccgttatcaacttgaaaaagtggcaccgagtcggtgc

SEQ ID NO: 151 - DNA, 76 bp, Artificial Sequence
  Guide RNA Scaffold v2
gttttagagctagaaatagcaagttaaaataaggctagtccgttatcaacttgaaaaagtggcaccgagtcggtgc

SEQ ID NO: 152 - DNA, 86 bp, Artificial Sequence
  Guide RNA Scaffold v3
gtttaagagctatgctggaaacagcatagcaagtttaaataaggctagtccgttatcaacttgaaaaagtggcaccgagtcggtgc